European Patent Application EP 4 678 187 A1, published January 14, 2026. Title: Compound for use in the treatment of inflammatory bowel disease. Applicant: Medizinische Hochschule Hannover. The sequence listing filed with the application follows.

SEQUENCE LISTING (74 sequences)

SEQ ID NO: 1 - protein, 248 aa, synthetic construct
  CHAIN 1..248: note = scFv MRU53-F8
QVQLQESGGGLVQPGRSLRLSCTASGFTFGDYAMSWVRQAPGKGLEWVGFIRSKAYGGTTEYAASVKGRFTISRDDSKSIAYLQMNSLKTEDTAVYYCTRVGGPDYGDPFDYWGQGTLVTVSSGSASAPKLEEGEFSEARVDIVMTQSPSSLSASVGDRATITCRASQSINNYLNWYQQKPGKAPNLLIYGASNLQGGVPSRFSGSGSGTDFTLTINSLQPEDFASYYCQQTYNTPITFGQGTRLEII

SEQ ID NO: 2 - protein, 280 aa, synthetic construct
  CHAIN 1..22: note = secretory signal
  CHAIN 23..47: note = VH FR1
  CHAIN 48..55: note = VH CDR1
  CHAIN 56..72: note = VH FR2
  CHAIN 73..82: note = VH CDR2
  CHAIN 83..120: note = VH FR3
  CHAIN 121..134: note = VH CDR3
  CHAIN 135..145: note = VH FR4
  CHAIN 164..189: note = VL FR1
  CHAIN 196..212: note = VL FR2
  CHAIN 213..215: note = VL CDR2
  CHAIN 216..251: note = VL FR3
  CHAIN 252..260: note = VL CDR3
  CHAIN 261..270: note = VL FR4
  CHAIN 271..280: note = VL linker
MKYLLPTAAAGLLLLAAQPAMAQVQLQESGGGLVQPGRSLRLSCTASGFTFGDYAMSWVRQAPGKGLEWVGFIRSKAYGGTTEYAASVKGRFTISRDDSKSIAYLQMNSLKTEDTAVYYCTRVGGPDYGDPFDYWGQGTLVTVSSGSASAPKLEEGEFSEARVDIVMTQSPSSLSASVGDRATITCRASQSINNYLNWYQQKPGKAPNLLIYGASNLQGGVPSRFSGSGSGTDFTLTINSLQPEDFASYYCQQTYNTPITFGQGTRLEIIRTVAAPSVAA

SEQ ID NO: 3 - protein, 246 aa, synthetic construct
  CHAIN 1..246: note = scFv MRU53-H1
QVQLQQSGGGLVQPGRSLGLSCTASGFTFGDYAMSWVRQAPGKGLEWVGFIRSKAYGGTTEYAASVKGRFTISRDDSESIAYLQMNSLKTEDTAVYYCTRGSYYSDAFDIWGQGTMVTVSSGSASAPKLEEGEFSEARVDIVLTQSPPSLSASVGDRVTITCRTSQSISSYLNWYQQKPGKAPKLLIYGASSLQSGVPSRFSGSGSGTDFTLTISSLQPEDFATFYCQQSYSSPPTFGQGTKVDIK

SEQ ID NO: 4 - protein, 278 aa, synthetic construct
  CHAIN 1..22: note = secretory signal
  CHAIN 23..47: note = VH FR1
  CHAIN 48..55: note = VH CDR1
  CHAIN 56..72: note = VH FR2
  CHAIN 73..82: note = VH CDR2
  CHAIN 83..120: note = VH FR3
  CHAIN 121..132: note = VH CDR3
  CHAIN 133..143: note = VH FR4
  CHAIN 162..187: note = VL FR1
  CHAIN 188..193: note = VL CDR1
  CHAIN 194..210: note = VL FR2
  CHAIN 211..213: note = VL CDR2
  CHAIN 214..249: note = VL FR3
  CHAIN 250..258: note = VL CDR3
  CHAIN 259..268: note = VL FR4
  CHAIN 269..278: note = VL linker
MKYLLPTAAAGLLLLAAQPAMAQVQLQQSGGGLVQPGRSLGLSCTASGFTFGDYAMSWVRQAPGKGLEWVGFIRSKAYGGTTEYAASVKGRFTISRDDSESIAYLQMNSLKTEDTAVYYCTRGSYYSDAFDIWGQGTMVTVSSGSASAPKLEEGEFSEARVDIVLTQSPPSLSASVGDRVTITCRTSQSISSYLNWYQQKPGKAPKLLIYGASSLQSGVPSRFSGSGSGTDFTLTISSLQPEDFATFYCQQSYSSPPTFGQGTKVDIKRTVAAPSVAA

SEQ ID NO: 5 - protein, 246 aa, synthetic construct
  CHAIN 1..246: note = scFv MRU54-A1
QVQLVQSGGGLVQPGRSLRLSCTASGFTFGDYAMSWVRQAPGKGLEWVGFIRSKAYGGTTEYAASVKGRFTISRDDSKSIAYLQMNSLKTEDTAVYYCTRAVEMADAFDIWGQGTMVTVSSGSASAPKLEEGEFSEARVDVVMTQSPSSLSASVGDRVTITCRASQSISSYLNWYQQKPGKAPKLLIYAASSLQSGVPSRFSGSGSGTDFTLTISSLQPEDFATYYCQQSYSTPFTFGPGTKVDIK

SEQ ID NO: 6 - protein, 278 aa, synthetic construct
  CHAIN 1..22: note = secretory signal
  CHAIN 23..47: note = VH FR1
  CHAIN 48..55: note = VH CDR1
  CHAIN 56..72: note = VH FR2
  CHAIN 73..82: note = VH CDR2
  CHAIN 83..120: note = VH FR3
  CHAIN 121..132: note = VH CDR3
  CHAIN 133..143: note = VH FR4
  CHAIN 162..187: note = VL FR1
  CHAIN 188..193: note = VL CDR1
  CHAIN 194..210: note = VL FR2
  CHAIN 211..213: note = VL CDR2
  CHAIN 214..249: note = VL FR3
  CHAIN 250..258: note = VL CDR3
  CHAIN 259..268: note = VL FR4
  CHAIN 269..278: note = VL linker
MKYLLPTAAAGLLLLAAQPAMAQVQLVQSGGGLVQPGRSLRLSCTASGFTFGDYAMSWVRQAPGKGLEWVGFIRSKAYGGTTEYAASVKGRFTISRDDSKSIAYLQMNSLKTEDTAVYYCTRAVEMADAFDIWGQGTMVTVSSGSASAPKLEEGEFSEARVDVVMTQSPSSLSASVGDRVTITCRASQSISSYLNWYQQKPGKAPKLLIYAASSLQSGVPSRFSGSGSGTDFTLTISSLQPEDFATYYCQQSYSTPFTFGPGTKVDIKRTVAAPSVAA

SEQ ID NO: 7 - protein, 247 aa, synthetic construct
  CHAIN 1..247: note = scFv UK013-B5
QVQLVQSGAEVRKSGESLKISCEGSGYSFGNYWIAWVRQMPGKGLEWMGIIYPGDSDTRYSPSFQGQVTISADKSISTAYLQWNTLKASDTAMYFCARHVDSTWYIDHWGQGTLVTVSSGSASAPKLEEGEFSEARVQPVLTQPPSASGSPGQSVTISCTGTSSDVGGYNFVSWYQHHPGKAPKLMIYEVSKRPSGVPDRFSASKSGNTASLTVSGLQADDEADYYCSSYAGNDNLQFGGGTKLTVL

SEQ ID NO: 8 - protein, 287 aa, synthetic construct
  CHAIN 1..22: note = secretory signal
  CHAIN 23..47: note = VH FR1
  CHAIN 48..55: note = VH CDR1
  CA_BIND 56..72: note = VH FR2
  CHAIN 73..80: note = VH CDR2
  CHAIN 81..118: note = VH FR3
  CHAIN 119..130: note = VH CDR3
  CHAIN 131..141: note = VH FR4
  CHAIN 160..184: note = VL FR1
  CHAIN 185..193: note = VL CDR1
  CHAIN 194..210: note = VL FR2
  CHAIN 211..213: note = VL CDR2
  CHAIN 214..249: note = VL FR3
  CHAIN 250..259: note = VL CDR3
  CHAIN 260..269: note = VL FR4
  CHAIN 270..287: note = VL linker
MKYLLPTAAAGLLLLAAQPAMAQVQLVQSGAEVRKSGESLKISCEGSGYSFGNYWIAWVRQMPGKGLEWMGIIYPGDSDTRYSPSFQGQVTISADKSISTAYLQWNTLKASDTAMYFCARHVDSTWYIDHWGQGTLVTVSSGSASAPKLEEGEFSEARVQPVLTQPPSASGSPGQSVTISCTGTSSDVGGYNFVSWYQHHPGKAPKLMIYEVSKRPSGVPDRFSASKSGNTASLTVSGLQADDEADYYCSSYAGNDNLQFGGGTKLTVLGRPKAAPSVTLFPPSSAA

SEQ ID NO: 9 - protein, 248 aa, synthetic construct
  CHAIN 1..248: note = scFv UK013-D5
QVQLQQSGAEVKKPGESLKISCEGSGYSFSNYWIAWVRQMPGKGLEWMGVIYPGDSDTRYSPSFQGQVTISADKSISTAYLQWSSLKASDTAMYYCARPPVGATDAFDIWGQGTMVTVSSGSASAPKLEEGEFSEARVQSALTQPPSASGSPGQSVTISCTGTSSDVGGYNFVSWYQQHPGKAPKLMIYEVSKRPSGVPDRFSGSKSGNTASLTVSGLQAEDEADYYCSSYAGSNNYVFGTGTKVTVL

SEQ ID NO: 10 - protein, 288 aa, synthetic construct
  CHAIN 1..22: note = secretory signal
  CHAIN 23..47: note = VH FR1
  CHAIN 48..55: note = VH CDR1
  CHAIN 56..72: note = VH FR2
  CHAIN 73..80: note = VH CDR2
  CHAIN 81..118: note = VH FR3
  CHAIN 119..131: note = VH CDR3
  CHAIN 132..142: note = VH FR4
  CHAIN 161..185: note = VL FR1
  CHAIN 186..194: note = VL CDR1
  CHAIN 194..211: note = VL FR2
  CHAIN 212..214: note = VL CDR2
  CHAIN 215..250: note = VL FR3
  CHAIN 251..260: note = VL CDR3
  CHAIN 261..270: note = VL FR4
  CHAIN 271..288: note = VL linker
MKYLLPTAAAGLLLLAAQPAMAQVQLQQSGAEVKKPGESLKISCEGSGYSFSNYWIAWVRQMPGKGLEWMGVIYPGDSDTRYSPSFQGQVTISADKSISTAYLQWSSLKASDTAMYYCARPPVGATDAFDIWGQGTMVTVSSGSASAPKLEEGEFSEARVQSALTQPPSASGSPGQSVTISCTGTSSDVGGYNFVSWYQQHPGKAPKLMIYEVSKRPSGVPDRFSGSKSGNTASLTVSGLQAEDEADYYCSSYAGSNNYVFGTGTKVTVLGQPKANPTVTLFPPSSAA

SEQ ID NO: 11 - protein, 248 aa, synthetic construct
  CHAIN 1..248: note = scFv UK013-F8
QVQLQESGGGLVKPGGSLRLSCAASGFTFSSYSMNWVRQAPGKGLEWVSSISSSSYIYYADSVKGRFTISRDNAKNSLYLQMNSLRAEDTAVYYCARREGGKYYYGMDVWGQGTTVTVSSGSASAPKLEEGEFSEARVQSALTQPPSASGSPGQSVTISCTGTSSDVGAYNYVSWYQQHPGKAPKLMIYEVTERPSGVPDRFSGSKSGNTASLTISGLQAEDEADYYCSSYTTSSTVLFGGGTKLTVL

SEQ ID NO: 12 - protein, 288 aa, synthetic construct
  CHAIN 1..22: note = secretory signal
  CHAIN 23..47: note = VH FR1
  CHAIN 48..55: note = VH CDR1
  CHAIN 56..72: note = VH FR2
  CHAIN 73..79: note = VH CDR2
  CHAIN 80..117: note = VH FR3
  CHAIN 118..131: note = VH CDR3
  CHAIN 132..142: note = VH FR4
  CHAIN 161..185: note = VL FR1
  CHAIN 186..194: note = VL CDR1
  CHAIN 195..211: note = VL FR2
  CHAIN 212..214: note = VL CDR2
  CHAIN 215..250: note = VL FR3
  CHAIN 251..260: note = VL CDR3
  CHAIN 261..270: note = VL FR4
  CHAIN 271..288: note = VL linker
MKYLLPTAAAGLLLLAAQPAMAQVQLQESGGGLVKPGGSLRLSCAASGFTFSSYSMNWVRQAPGKGLEWVSSISSSSYIYYADSVKGRFTISRDNAKNSLYLQMNSLRAEDTAVYYCARREGGKYYYGMDVWGQGTTVTVSSGSASAPKLEEGEFSEARVQSALTQPPSASGSPGQSVTISCTGTSSDVGAYNYVSWYQQHPGKAPKLMIYEVTERPSGVPDRFSGSKSGNTASLTISGLQAEDEADYYCSSYTTSSTVLFGGGTKLTVLGQPKAAPSVTLFPPSSAA

SEQ ID NO: 13 - protein, 254 aa, synthetic construct
  CHAIN 1..254: note = scFv UK013-H4
QVQLQESGGGVVQPGRSLRLSCAASGFTFSSYAMHWVRQAPGKGLEWVAVISYDGSNKYYADSVKGRFTISRDNSKNTLYLQMNSLRAEDTAVYYCARAPYYYDTPRTYYYGMDVWGQGTTVTVSSGSASAPKLEEGEFSEARVSYELTQPPSASGTPGQTFTISCSGSDSNIERNFVYWYQQLPGTAPKLLIYRTDQRPSGVPDRFSGSKSGSSASLAISGLRSEDEAHYYCSTWDDSLTGVVFGGGTKLTVL

SEQ ID NO: 14 - protein, 294 aa, synthetic construct
  CHAIN 1..22: note = secretory signal
  CHAIN 23..47: note = VH FR1
  CHAIN 48..55: note = VH CDR1
  CHAIN 56..72: note = VH FR2
  CHAIN 73..80: note = VH CDR2
  CHAIN 81..118: note = VH FR3
  CHAIN 138..148: note = VH FR4
  CHAIN 167..191: note = VL FR1
  CHAIN 192..199: note = VL CDR1
  CHAIN 200..216: note = VL FR2
  CHAIN 217..219: note = VL CDR2
  CHAIN 220..255: note = VL FR3
  CHAIN 256..266: note = VL CDR3
  CHAIN 267..276: note = VL FR4
  CHAIN 119..137: note = VH CDR3
  CHAIN 277..294: note = VL linker
MKYLLPTAAAGLLLLAAQPAMAQVQLQESGGGVVQPGRSLRLSCAASGFTFSSYAMHWVRQAPGKGLEWVAVISYDGSNKYYADSVKGRFTISRDNSKNTLYLQMNSLRAEDTAVYYCARAPYYYDTPRTYYYGMDVWGQGTTVTVSSGSASAPKLEEGEFSEARVSYELTQPPSASGTPGQTFTISCSGSDSNIERNFVYWYQQLPGTAPKLLIYRTDQRPSGVPDRFSGSKSGSSASLAISGLRSEDEAHYYCSTWDDSLTGVVFGGGTKLTVLGQPKAAPSVTLFPPSSAA

SEQ ID NO: 15 - protein, 241 aa, synthetic construct
  CHAIN 1..241: note = UK027-F5
QVQLVQSGAEVKKPGASVKVSCKASGYTFTGYYMHWVRQAPGQGLEWMGWINPNSGGTNYAQKFQGRVTMTRDTSISTAYMELSRLRSDDTAVYYCARAPFGSADYWGQGTLVTVSSGSASAPKLEEGEFSEARVQPVLTQPPSVSVSPXQTASISCSGDRLGDKYVAWYQQKAGQSPVLVIYADAKRPSGIPERFSGSNSGNTATLTISGTQALDEGDYYCQAWDTFTVIFGGGTKLTVL

SEQ ID NO: 16 - protein, 281 aa, synthetic construct
  CHAIN 1..22: note = secretory signal
  CHAIN 23..47: note = VH FR1
  CA_BIND 48..55: note = VH CDR1
  CHAIN 56..72: note = VH FR2
  CHAIN 73..80: note = VH CDR2
  CHAIN 81..118: note = VH FR3
  CHAIN 119..128: note = VH CDR3
  CHAIN 129..139: note = VH FR4
  CHAIN 158..182: note = VL FR1
  CHAIN 183..188: note = VL CDR1
  CHAIN 189..205: note = VL FR2
  CHAIN 206..208: note = VL CDR2
  CHAIN 209..244: note = VL FR3
  CHAIN 245..253: note = VL CDR3
  CHAIN 254..263: note = VL FR4
  CHAIN 264..281: note = VL linker
MKYLLPTAAAGLLLLAAQPAMAQVQLVQSGAEVKKPGASVKVSCKASGYTFTGYYMHWVRQAPGQGLEWMGWINPNSGGTNYAQKFQGRVTMTRDTSISTAYMELSRLRSDDTAVYYCARAPFGSADYWGQGTLVTVSSGSASAPKLEEGEFSEARVQPVLTQPPSVSVSPXQTASISCSGDRLGDKYVAWYQQKAGQSPVLVIYADAKRPSGIPERFSGSNSGNTATLTISGTQALDEGDYYCQAWDTFTVIFGGGTKLTVLGQPKAAPSVTLFPPSSAA

SEQ ID NO: 17 - protein, 22 aa, synthetic construct
  CHAIN 1..22: note = secretory signal, murine
MDFQVQIFSFLLISASVIMSRT

SEQ ID NO: 18 - protein, 21 aa, synthetic construct
  CHAIN 1..21: note = secretory signal, murine
MWWRLWWLLLLLLLLWPMVWA

SEQ ID NO: 19 - protein, 20 aa, synthetic construct
  CHAIN 1..20: note = secretory signal, human
MWWRLWWLLLLLLLLWPMVW

SEQ ID NO: 20 - protein, 21 aa, synthetic construct
  CHAIN 1..21: note = secretory signal, human
MDFQVQIFSFLLISASVIMSR

SEQ ID NO: 21 - protein, 226 aa, synthetic construct
VPRDGGCKPCICTVPEVSSVFIFPPKPKDVLTITLTPKVTCVVVDISKDDPEVQFSWFVDDVEVHTAQTQPREEQFNSTFRSVSELPIMHQDWLNGKEFKCRVNSAAFPAPIEKTISKTKGRPKAPQVCTIPPPKEQMAKDKVSLTCMITDFFPEDITVEWQWNGQPAENYKNTQPIMDTDGSYFVYSKLNVQKSNWEAGNTFTCSVLHEGLHNHHTEKSLSHSPG

SEQ ID NO: 22 - protein, 58 aa, synthetic construct
FSSVVPVLQKVNSTTTKPVLRTPSPVHPTGTSQPQRPEDCRPRGSVKGTGLDFACDIY

SEQ ID NO: 23 - protein, 83 aa, synthetic construct
FVPVFLPAKPTTTPAPRPPTPAPTIASQPLSLRPEASRPAAGGAVHTRGLDFADIYIWAPLAGTCGVLLLSLVITLYCNHRQL

SEQ ID NO: 24 - protein, 234 aa, synthetic construct
PAEPKSPDKTHTCPPCPAPPVAGPSVFLFPPKPKDTLMIARTPEVTCVVVDVSHEDPEVKFNWYVDGVEVHNAKTKPREEQYNSTYRVVSVLTVLHQDWLNGKEYKCKVSNKALPAPIEKTISKAKGQPREPQVYTLPPSRDELTKNQVSLTCLVKGFYPSDIAVEWESNGQPENNYKTTPPVLDSDGSFFLYSKLTVDKSRWQQGNVFSCSVMHEALHNHYTQKSLSLSPGKK

SEQ ID NO: 25 - protein, 25 aa, synthetic construct
VFLACVLGGSFGFLGFLGLCILCCV

SEQ ID NO: 26 - protein, 25 aa, synthetic construct
IWAPLAGICVALLLSLIITLICYHR

SEQ ID NO: 27 - protein, 45 aa, synthetic construct
QLWTNSRRNRLLQSDYMNMTPRRPGLTRKPYQPYAPARDFAAYRP

SEQ ID NO: 28 - protein, 113 aa, synthetic construct
RAKFSRSAETAANLQDPNQLYNELNLGRREEYDVLEKKRARDPEMGGKQQRRRNPQEGVYNALQKDKMAEAYSEIGTKGERRRGKGHDGLYQGLSTATKDTYDALHMQTLAPR

SEQ ID NO: 29 - protein, 43 aa, synthetic construct
WTNSRRNRLLQSDYMNMTPRRPGLTRKPYQPYAPARDFAAYRP

SEQ ID NO: 30 - protein, 113 aa, synthetic construct; identical to SEQ ID NO: 28

SEQ ID NO: 31 - protein, 43 aa, synthetic construct
WVRSKRSRLLHSDYMNMTPRRPGPTRKHYQPYAPPRDFAAYRS

SEQ ID NO: 32 - protein, 115 aa, synthetic construct
RVKFSRSADAPAYQQGQNQLYNELNLGRREEYDVLDKRRGRDPEMGGKPRRKNPQEGLYNELQKDKMAEAYSEIGMKGERRRGKGHDGLYQGLSTATKDTYDALHMQALPPRSSR

SEQ ID NO: 33 - protein, 72 aa, synthetic construct
DPKFWVLVVVGGVLACYSLLVTVAFIIFWVRSKRSRLLHSDYMNMTPRRPGPTRKHYQAYAAARDFAAYRSL

SEQ ID NO: 34 - protein, 112 aa, synthetic construct
RVKFSRSADAPAYQQGQNQLYNELNLGRREEYDVLDKRRGRDPEMGGKPRRKNPQEGLYNELQKDKMAEAYSEIGMKGERRRGKGHDGLYQGLSTATKDTYDALHMQALPPR

SEQ ID NO: 35 - protein, 19 aa, synthetic construct
ATNFSLLKQAGDVEENPGP

SEQ ID NO: 36 - protein, 429 aa, synthetic construct
MPNPRPAKPMAPSLALGPSPGVLPSWKTAPKGSELLGTRGSGGPFQGRDLRSGAHTSSSLNPLPPSQLQLPTVPLVMVAPSGARLGPSPHLQALLQDRPHFMHQLSTVDAHAQTPVLQVRPLDNPAMISLPPPSAATGVFSLKARPGLPPGINVASLEWVSREPALLCTFPRSGTPRKDSNLLAAPQGSYPLLANGVCKWPGCEKVFEEPEEFLKHCQADHLLDEKGKAQCLLQREVVQSLEQQLELEKEKLGAMQAHLAGKMALAKAPSVASMDKSSCCIVATSTQGSVLPAWSAPREAPDGGLFAVRRHLWGSHGNSSFPEFFHNMDYFKYHNMRPPFTYATLIRWAILEAPERQRTLNEIYHWFTRMFAYFRNHPATWKNAIRHNLSLHKCFVRVESEKGAVWTVDEFEFRKKRSQRPNKCSNPCP

SEQ ID NO: 37 - protein, 449 aa, synthetic construct
ATNFSLLKQAGDVEENPGPSMPNPRPAKPMAPSLALGPSPGVLPSWKTAPKGSELLGTRGSGGPFQGRDLRSGAHTSSSLNPLPPSQLQLPTVPLVMVAPSGARLGPSPHLQALLQDRPHFMHQLSTVDAHAQTPVLQVRPLDNPAMISLPPPSAATGVFSLKARPGLPPGINVASLEWVSREPALLCTFPRSGTPRKDSNLLAAPQGSYPLLANGVCKWPGCEKVFEEPEEFLKHCQADHLLDEKGKAQCLLQREVVQSLEQQLELEKEKLGAMQAHLAGKMALAKAPSVASMDKSSCCIVATSTQGSVLPAWSAPREAPDGGLFAVRRHLWGSHGNSSFPEFFHNMDYFKYHNMRPPFTYATLIRWAILEAPERQRTLNEIYHWFTRMFAYFRNHPATWKNAIRHNLSLHKCFVRVESEKGAVWTVDEFEFRKKRSQRPNKCSNPCP

SEQ ID NO: 38 - protein, 431 aa, synthetic construct
MPNPRPGKPSAPSLALGPSPGASPSWRAAPKASDLLGARGPGGTFQGRDLRGGAHASSSSLNPMPPSQLQLPTLPLVMVAPSGARLGPLPHLQALLQDRPHFMHQLSTVDAHARTPVLQVHPLESPAMISLTPPTTATGVFSLKARPGLPPGINVASLEWVSREPALLCTFPNPSAPRKDSTLSAVPQSSYPLLANGVCKWPGCEKVFEEPEDFLKHCQADHLLDEKGRAQCLLQREMVQSLEQQLVLEKEKLSAMQAHLAGKMALTKASSVASSDKGSCCIVAAGSQGPVVPAWSGPREAPDSLFAVRRHLWGSHGNSTFPEFLHNMDYFKFHNMRPPFTYATLIRWAILEAPEKQRTLNEIYHWFTRMFAFFRNHPATWKNAIRHNLSLHKCFVRVESEKGAVWTVDELEFRKKRSQRPSRCSNPTPGP

SEQ ID NO: 39 - DNA, 4899 bp, synthetic construct
  source 1..4899: mol_type = other DNA
  CDS 1..840: note = secretory signal - scFv MRU53-F8; protein_id = 43; translation = MKYLLPTAAAGLLLLAAQPAMAQVQLQESGGGLVQPGRSLRLSCTASGFTFGDYAMSWVRQAPGKGLEWVGFIRSKAYGGTTEYAASVKGRFTISRDDSKSIAYLQMNSLKTEDTAVYYCTRVGGPDYGDPFDYWGQGTLVTVSSGSASAPKLEEGEFSEARVDIVMTQSPSSLSASVGDRATITCRASQSINNYLNWYQQKPGKAPNLLIYGASNLQGGVPSRFSGSGSGTDFTLTINSLQPEDFASYYCQQTYNTPITFGQGTRLEIIRTVAAPSVAA
  CDS 841..849: note = linker; translation = APA
  CDS 850..1542: note = hIgG hinge; protein_id = 44; translation = EPKSPDKTHTCPPCPAPPVAGPSVFLFPPKPKDTLMIARTPEVTCVVVDVSHEDPEVKFNWYVDGVEVHNAKTKPREEQYNSTYRVVSVLTVLHQDWLNGKEYKCKVSNKALPAPIEKTISKAKGQPREPQVYTLPPSRDELTKNQVSLTCLVKGFYPSDIAVEWESNGQPENNYKTTPPVLDSDGSFFLYSKLTVDKSRWQQGNVFSCSVMHEALHNHYTQKSLSLSPGK
  CDS 1543..1641: note = hCD28 TM; protein_id = 45; translation = KQLDPKFWVLVVVGGVLACYSLLVTVAFIIFWV
  CDS 1642..1764: note = hCD28 ICD; protein_id = 46; translation = RSKRSRLLHSDYMNMTPRRPGPTRKHYQAYAAARDFAAYRS
  CDS 1765..1767: note = linker; translation = L
  CDS 1768..2103: note = hCD3zeta ICD; protein_id = 47; translation = RVKFSRSADAPAYQQGQNQLYNELNLGRREEYDVLDKRRGRDPEMGGKPRRKNPQEGLYNELQKDKMAEAYSEIGMKGERRRGKGHDGLYQGLSTATKDTYDALHMQALPPR
  CDS 2104..2112: note = linker; translation = SRG
  CDS 2113..2169: note = P2A site; protein_id = 48; translation = ATNFSLLKQAGDVEENPGP
  CDS 2170..2172: note = linker; translation = S
  CDS 2173..3468: map = human FOXP3; protein_id = 49; translation = MPNPRPGKPSAPSLALGPSPGASPSWRAAPKASDLLGARGPGGTFQGRDLRGGAHASSSSLNPMPPSQLQLPTLPLVMVAPSGARLGPLPHLQALLQDRPHFMHQLSTVDAHARTPVLQVHPLESPAMISLTPPTTATGVFSLKARPGLPPGINVASLEWVSREPALLCTFPNPSAPRKDSTLSAVPQSSYPLLANGVCKWPGCEKVFEEPEDFLKHCQADHLLDEKGRAQCLLQREMVQSLEQQLVLEKEKLSAMQAHLAGKMALTKASSVASSDKGSCCIVAAGSQGPVVPAWSGPREAPDSLFAVRRHLWGSHGNSTFPEFLHNMDYFKFHNMRPPFTYATLIRWAILEAPEKQRTLNEIYHWFTRMFAFFRNHPATWKNAIRHNLSLHKCFVRVESEKGAVWTVDELEFRKKRSQRPSRCSNPTPGP
  primer_bind 3469..4050: note = IRES
  misc_feature 4051..4056: note = DNA linker
  CDS 4057..4899: note = deltaLNGFR; protein_id = 50; translation = MGAGATGRAMDGPRLLLLLLLGVSLGGAKEACPTGLYTHSGECCKACNLGEGVAQPCGANQTVCEPCLDSVTFSDVVSATEPCKPCTECVGLQSMSAPCVEADDAVCRCAYGYYQDETTGRCEACRVCEAGSGLVFSCQDKQNTVCEECPDGTYSDEANHVDPCLPCTVCEDTERQLRECTRWADAECEEIPGRWITRSTPPEGSDSTAPSTQEPEAPPEQDLIASTVAGVVTTVMGSSQPVVTRGTTDNLIPVYCSILAAVVVGLVAYIAFKRWNRGIL
atgaaatacctattgcctacggcagccgctggcttgctgctgctggcagctcagccggccatggcccaggtgcaactgcaggagtcggggggaggcttggtacagccagggcggtccctgagactctcctgtacagcttctggattcacctttggtgattatgctatgagctgggtccgccaggctccagggaaggggctggagtgggtaggtttcattagaagcaaagcttatggtgggacaacagaatacgccgcgtctgtgaaaggcagattcaccatctcaagagatgattccaaaagcatcgcctatctgcaaatgaacagcctgaaaaccgaggacacagccgtgtattactgtactagagtcggggggcctgattacggtgatccgtttgactactggggccagggaaccctggtcaccgtctcctcagggagtgcatccgccccaaagcttgaagaaggtgaattttcagaagcacgcgtagacatcgtgatgacccagtctccatcctccctgtctgcgtctgtaggagacagagccaccatcacttgccgggcaagtcagagcattaacaattatttaaattggtatcagcagaaaccagggaaagcccctaacctcctgatctatggtgcatccaatttgcaaggtggggtcccatcaaggttcagtggcagtggatctgggacagatttcactctcaccatcaacagtctgcaacctgaagattttgcaagttactactgtcaacagacttacaatactccgatcaccttcggccaagggacacgactggaaattatacgaactgtggctgcaccatctgtcgcggccgcaccagccgagcctaagagccctgataagacccacacctgtcctccatgtcctgctcctccagtggctggcccttccgtgtttctgttccctccaaagcctaaggacaccctgatgatcgccagaacacccgaagtgacctgcgtggtggtggatgtgtcccacgaagatcctgaagtgaagtttaattggtacgtggacggcgtggaagtgcacaacgccaagaccaagcctagagaggaacagtacaacagcacctacagagtggtgtccgtgctgaccgtgctgcaccaggattggctgaacggcaaagagtacaagtgcaaggtgtccaacaaggccctgcctgctcctatcgaaaagaccatcagcaaggccaagggacagcccagagaaccccaggtgtacacactgcctccaagcagagatgagctgaccaagaaccaggtgtccctgacctgtctggtcaagggcttctacccctccgatatcgccgtggaatgggagagcaatggccagccagagaacaactacaagaccacacctcctgtgctggactccgatggctcattcttcctgtacagcaagctgacagtggacaagagcagatggcagcagggcaacgtgttcagctgcagcgtgatgcacgaggccctgcacaaccactacacccagaagtccctgtctctgagccccggcaagaagcaattggaccccaagttctgggtgctcgtggtcgttggaggcgtgctggcctgttatagcctgctggttaccgtggcctttatcatcttctgggtccgaagcaagcggagcagactgctgcacagcgactacatgaacatgacccctagacggcccggacctaccagaaagcactatcaggcctatgccgccgctagagatttcgccgcctacagatccctgcgcgtgaagttcagcagatccgccgatgctcctgcctatcagcagggccagaatcagctgtacaacgagctgaatctggggcgcagagaagagtacgacgtgctggataagcggagaggcagagatcctgagatgggcggcaagcccagacggaagaatcctcaagagggcctgtataatgagctgcagaaagacaagatggccgaggcctacagcgagatcggaatgaagggcgaacgcagaagaggcaagggccacgatggactgtatcagggcctgagcaccgccaccaaggacacatatgacgcactgcacatgcaggctctgcctccacgatctagaggagccaccaacttctccctgctgaagcaggccggcgacgtggaggagaaccccggcccctctatgcctaatcctagacctggaaagcccagcgcacctagccttgctcttggaccttctcctggcgcctctccatcttggagagccgctcctaaagccagcgatctgctcggagctagaggacctggcggcacatttcagggaagagatctgagaggcggagcccacgctagcagtagctccctgaatcctatgcctcctagccagctccagctgcctacactgccactggttatggtggcacctagcggcgctagacttggcccactgcctcatcttcaagctctgctgcaggacagaccccacttcatgcaccagctgtccaccgtggatgcccacgcaagaacacctgtgctgcaggttcaccctctggaatccccagccatgatcagcctgacacctccaacaacagccaccggcgtgttctccctgaaagccagacctggactgcctcctggcatcaatgtggctagcctggaatgggtgtcccgcgaacctgctctgctgtgcacattccccaatcctagcgctcccagaaaggacagcacactgtctgccgtgcctcagagcagctatcccctgcttgctaacggcgtgtgcaagtggcctggatgcgagaaggtgttcgaggaacccgaggacttcctgaagcactgccaggccgatcatctgctggacgaaaagggcagagcccagtgtctgctccagcgcgaaatggtgcagtccctggaacagcagctggtcctggaaaaagaaaagctgagcgccatgcaggcccacctggccggaaaaatggccctgacaaaagccagcagcgtggccagctctgataagggcagctgttgtatcgtggccgctggatctcagggaccagtggtgccagcttggagcggacctagagaagcccctgatagcctgtttgccgtgcggagacatctgtggggctctcacggcaactctactttccccgagttcctgcacaatatggactacttcaagttccacaacatgcggcctccattcacctacgccacactgatcagatgggccatcctggaagccccagagaagcagagaacactgaacgagatctaccactggtttacccggatgttcgccttctttcggaatcaccccgccacctggaagaacgccatcagacacaatctgagcctgcacaagtgcttcgtgcgcgtggaatctgagaaaggcgccgtgtggactgtggacgagctggaattccgcaagaaaagaagccagcggcctagccggtgcagcaacccaacacctggaccttaatctagatgacccctctccctcccccccccctaacgttactggccgaagccgcttggaataaggccggtgtgcgtttgtctatatgttattttccaccatattgccgtcttttggcaatgtgaggccccggaaacctggccctgtcttcttgacgagcattcctaggggtctttcccctctcgccaaaggaatgcaaggtctgttgaatgtcgtgaaggaagcagttcctctggaagcttcttgaagacaaacaacgtctgtagcgaccctttgcaggcagcggaaccccccacctggcgacaggtgcctctgcggccaaaagccacgtgtataagatacacctgcaaaggcggcacaaccccagtgccacgttgtgagttggatagttgtggaaagagtcaaatggctctcctcaagcgtattcaacaaggggctgaaggatgcccagaaggtaccccattgtatgggatctgatctggggcctcggtgcacatgctttacatgtgtttagtcgaggttaaaaaacgtctaggccccccgaaccacggggacgtggtttccctttgaaaaacacgataatactccggaatgggcgctggcgccacaggcagagctatggatggacctagactcctgctgctgctcctgctgggagtttctcttggcggagccaaagaggcctgtcctaccggactgtacacacactctggcgagtgctgcaaggcctgcaatctcggagaaggcgtggcacaaccttgcggcgcaaatcagaccgtgtgcgagccttgtctggatagcgtgaccttcagcgacgtggtgtctgccaccgagccttgcaagccttgtaccgagtgtgtgggactgcagagcatgagcgccccttgtgtggaagccgatgatgccgtgtgcagatgcgcctacggctactaccaggacgagacaacaggcagatgcgaggcctgtagagtgtgcgaagctggctctggactggtgttctcctgccaagacaagcagaacaccgtgtgtgaagagtgccccgacggcacctatagcgacgaagccaatcacgtggacccttgtctgccttgcacagtgtgcgaggacaccgagagacagctgcgcgagtgtactagatgggccgatgccgagtgcgaagagatccctggcagatggatcaccagaagcacaccacctgagggcagcgatagcacagccccttctacacaagagcccgaggctcctcctgagcaggatctgattgcctctacagtggccggcgtggtcaccacagtgatgggatcttctcagcccgtcgtgaccagaggcacaaccgacaatctgatccccgtgtactgcagcattctggccgccgtggttgtgggactcgtggcctatatcgccttcaagcggtggaaccggggcatcctctaa

SEQ ID NO: 40 - DNA, 4362 bp, synthetic construct
  source 1..4362: mol_type = other DNA
  CDS 1..840: note = secretory signal - scFv MRU53-F8; protein_id = 51; translation = MKYLLPTAAAGLLLLAAQPAMAQVQLQESGGGLVQPGRSLRLSCTASGFTFGDYAMSWVRQAPGKGLEWVGFIRSKAYGGTTEYAASVKGRFTISRDDSKSIAYLQMNSLKTEDTAVYYCTRVGGPDYGDPFDYWGQGTLVTVSSGSASAPKLEEGEFSEARVDIVMTQSPSSLSASVGDRATITCRASQSINNYLNWYQQKPGKAPNLLIYGASNLQGGVPSRFSGSGSGTDFTLTINSLQPEDFASYYCQQTYNTPITFGQGTRLEIIRTVAAPSVAA
  CDS 850..1008: note = human CD8 hinge; protein_id = 52; translation = FVPVFLPAKPTTTPAPRPPTPAPTIASQPLSLRPEASRPAAGGAVHTRGLDFA
  CDS 1009..1092: note = hCD8 TM; protein_id = 53; translation = DIYIWAPLAGTCGVLLLSLVITLYCNHR
  CDS 1093..1104: map = linker; protein_id = 54; translation = QLWV
  CDS 1105..1227: note = hCD28 ICD; protein_id = 55; translation = RSKRSRLLHSDYMNMTPRRPGPTRKHYQPYAPPRDFAAYRS
  CDS 1228..1563: note = hCD3 ICD; protein_id = 56; translation = RVKFSRSADAPAYQQGQNQLYNELNLGRREEYDVLDKRRGRDPEMGGKPRRKNPQEGLYNELQKDKMAEAYSEIGMKGERRRGKGHDGLYQGLSTATKDTYDALHMQALPPR
  CDS 1564..1575: note = linker; protein_id = 57; translation = SSRG
  CDS 1576..1632: note = P2A site; protein_id = 58; translation = ATNFSLLKQAGDVEENPGP
  CDS 1633..1635: note = linker; translation = S
  CDS 1636..2931: note = hFOXP3; protein_id = 59; translation = MPNPRPGKPSAPSLALGPSPGASPSWRAAPKASDLLGARGPGGTFQGRDLRGGAHASSSSLNPMPPSQLQLPTLPLVMVAPSGARLGPLPHLQALLQDRPHFMHQLSTVDAHARTPVLQVHPLESPAMISLTPPTTATGVFSLKARPGLPPGINVASLEWVSREPALLCTFPNPSAPRKDSTLSAVPQSSYPLLANGVCKWPGCEKVFEEPEDFLKHCQADHLLDEKGRAQCLLQREMVQSLEQQLVLEKEKLSAMQAHLAGKMALTKASSVASSDKGSCCIVAAGSQGPVVPAWSGPREAPDSLFAVRRHLWGSHGNSTFPEFLHNMDYFKFHNMRPPFTYATLIRWAILEAPEKQRTLNEIYHWFTRMFAFFRNHPATWKNAIRHNLSLHKCFVRVESEKGAVWTVDELEFRKKRSQRPSRCSNPTPGP
  primer_bind 2932..3510: note = IRES
  misc_feature 3511..3516: note = DNA linker
  CDS 3517..4362: note = deltaLNGFR; protein_id = 60; translation = GMGAGATGRAMDGPRLLLLLLLGVSLGGAKEACPTGLYTHSGECCKACNLGEGVAQPCGANQTVCEPCLDSVTFSDVVSATEPCKPCTECVGLQSMSAPCVEADDAVCRCAYGYYQDETTGRCEACRVCEAGSGLVFSCQDKQNTVCEECPDGTYSDEANHVDPCLPCTVCEDTERQLRECTRWADAECEEIPGRWITRSTPPEGSDSTAPSTQEPEAPPEQDLIASTVAGVVTTVMGSSQPVVTRGTTDNLIPVYCSILAAVVVGLVAYIAFKRWNRGIL
atgaaatacctattgcctacggcagccgctggcttgctgctgctggcagctcagccggccatggcccaggtgcaactgcaggagtcggggggaggcttggtacagccagggcggtccctgagactctcctgtacagcttctggattcacctttggtgattatgctatgagctgggtccgccaggctccagggaaggggctggagtgggtaggtttcattagaagcaaagcttatggtgggacaacagaatacgccgcgtctgtgaaaggcagattcaccatctcaagagatgattccaaaagcatcgcctatctgcaaatgaacagcctgaaaaccgaggacacagccgtgtattactgtactagagtcggggggcctgattacggtgatccgtttgactactggggccagggaaccctggtcaccgtctcctcagggagtgcatccgccccaaagcttgaagaaggtgaattttcagaagcacgcgtagacatcgtgatgacccagtctccatcctccctgtctgcgtctgtaggagacagagccaccatcacttgccgggcaagtcagagcattaacaattatttaaattggtatcagcagaaaccagggaaagcccctaacctcctgatctatggtgcatccaatttgcaaggtggggtcccatcaaggttcagtggcagtggatctgggacagatttcactctcaccatcaacagtctgcaacctgaagattttgcaagttactactgtcaacagacttacaatactccgatcaccttcggccaagggacacgactggaaattatacgaactgtggctgcaccatctgtcgcggccgcggccgcattcgtgcccgtgtttctgcctgccaagcctaccacaacacccgctcctagacctccaacaccagctccaacaatcgccagccagcctctgtctctgaggcctgaagctagcagacctgctgctggcggagccgtgcatacaagaggactggatttcgccgacatctacatctgggctcctctggccggaacatgcggagtgctgctgctcagcctggttatcaccctgtactgcaaccaccggcaattgtgggtccgaagcaagcggtccagactgctgcacagcgactacatgaacatgacccctagacggcccggacctaccagaaagcactaccagccttacgctcctcctagagactttgccgcctatcggagcagagtgaagttcagcagatccgccgatgctcccgcctatcagcagggacagaatcagctgtacaacgagctgaatctggggcgcagagaagagtacgacgtgctggacaagagaagaggcagggaccctgagatgggcggcaagcccagaagaaagaaccctcaagagggcctgtataatgagctgcagaaagacaagatggccgaggcctacagcgagatcggaatgaagggcgaacgcagaagaggaaagggccacgacggactgtatcagggcctgagcacagccacaaaggacacctatgacgccctgcacatgcaggccctgcctccaagatcttctagaggagccaccaacttctccctgctgaagcaggccggcgacgtggaggagaaccccggcccctctatgcctaatcctagaccaggcaagcctagcgctcctagccttgctcttggaccttctcctggcgcctctccatcttggagagccgctcctaaagccagcgatctgctcggagctagaggacctggcggcacatttcagggcagagatcttagaggcggagcccacgctagcagtagctccctgaatcctatgcctcctagccagctccagctgcctacactgcctctggttatggtggcacctagcggagcaagactgggacctctgccacatctgcaggctctgctgcaggacagaccccactttatgcaccagctgagcaccgtggatgcccacgcaagaacacctgtgctgcaggttcaccctctggaaagccccgccatgatcagcctgacaccacctacaacagccaccggcgtgttctccctgaaagccagacctggactgcctcctggcatcaatgtggctagcctggaatgggtgtcccgcgaacctgcactgctgtgcacattccccaatccaagcgctcccagaaaggacagcacactgtctgccgtgcctcagagcagctatcccctgcttgctaacggcgtgtgcaagtggcctggatgcgagaaggtgttcgaggaacccgaggacttcctgaagcactgccaggccgatcatctgctggacgaaaaaggcagagcccagtgtctgctccagcgcgagatggtgcagtctctggaacagcagctggtcctggaaaaagaaaagctgagcgccatgcaggctcacctggctggaaaaatggccctgacaaaggccagcagcgtggcctcttctgataagggcagctgctgcattgtggccgctggatctcagggacctgttgtgcctgcttggagcggacctagagaggcccctgattctctgtttgccgtgcggagacatctgtggggctctcacggcaactctactttccccgagttcctgcacaacatggactacttcaagttccacaacatgcggcctccattcacctacgccacactgatcagatgggccatcctggaagcccctgagaagcagagaaccctgaacgagatctaccactggtttacccggatgttcgccttctttcggaatcaccccgccacctggaagaacgccatcagacacaatctgagtctgcacaagtgcttcgtgcgcgtggaatctgagaaaggcgccgtgtggacagtggacgagctggaattcagaaagaagcggagccagcggcctagcagatgtagcaaccctacacctggaccttaatctagatgacccctctccctcccccccccctaacgttactggccgaagccgcttggaataaggccggtgtgcgtttgtctatatgttattttccaccatattgccgtcttttggcaatgtgaggccccggaaacctggccctgtcttcttgacgagcattcctaggggtctttcccctctcgccaaaggaatgcaaggtctgttgaatgtcgtgaaggaagcagttcctctggaagcttcttgaagacaaacaacgtctgtagcgaccctttgcaggcagcggaaccccccacctggcgacaggtgcctctgcggccaaaagccacgtgtataagatacacctgcaaaggcggcacaaccccagtgccacgttgtgagttggatagttgtggaaagagtcaaatggctctcctcaagcgtattcaacaaggggctgaaggatgcccagaaggtaccccattgtatgggatctgatctggggcctcggtgcacatgctttacatgtgtttagtcgaggttaaaaaacgtctaggccccccgaaccacggggacgtggtttccctttgaaaaacacgataatactccggaatgggcgctggcgccacaggcagagctatggatggacctagactgctcctcctgctgctcctgggagtttctctcggcggagccaaagaggcctgtcctaccggactgtacacacactctggcgagtgctgcaaggcctgcaatctcggagaaggcgtggcacaaccttgcggcgctaatcagaccgtgtgcgagccttgtctggactccgtgacctttagcgacgtggtgtctgccaccgagccttgcaagccttgtaccgagtgtgtgggcctgcagagcatgtctgccccttgtgtggaagccgacgatgccgtgtgtagatgcgcctacggctactaccaggacgagacaacaggcagatgcgaggcctgtagagtgtgcgaagctggctctggactggtgttcagctgccaagacaagcagaacaccgtgtgtgaagagtgccccgacggcacctatagcgacgaagccaatcacgtggacccctgcctgccttgtactgtgtgcgaggacaccgagcggcagctgagagaatgtactagatgggccgacgccgagtgcgaagagatccctggaagatggatcaccagaagcaccccacctgagggcagcgattctacagccccaagcacacaagagcccgaggctcctccagaacaggacctgattgcctctacagtggccggcgtcgtgacaacagtgatgggatcttctcagcccgtggtcaccaggggcaccaccgataatctgatccccgtgtactgcagcatcctggccgctgtggttgtgggactcgtggcctatatcgccttcaagcggtggaaccggggcatcctctaa

SEQ ID NO: 41 - DNA, 4032 bp, synthetic construct
  source 1..4032: mol_type = other DNA
  CDS 1..864: note = secretory signal - scFv UK017-F8; protein_id = 61; translation = MKYLLPTAAAGLLLLAAQPAMAQVQLQESGGGLVKPGGSLRLSCAASGFTFSSYSMNWVRQAPGKGLEWVSSISSSSYIYYADSVKGRFTISRDNAKNSLYLQMNSLRAEDTAVYYCARREGGKYYYGMDVWGQGTTVTVSSGSASAPKLEEGEFSEARVQSALTQPPSASGSPGQSVTISCTGTSSDVGAYNYVSWYQQHPGKAPKLMIYEVTERPSGVPDRFSGSKSGNTASLTISGLQAEDEADYYCSSYTTSSTVLFGGGTKLTVLGQPKAAPSVTLFPPSSAA
  CDS 1123..1179: note = murine CD28 ICD; protein_id = 62; translation = WTNSRRNRLLQSDYMNMTP
  CDS 865..1122: note = murine CD8 TM; protein_id = 63; translation = AFSSVVPVLQKVNSTTTKPVLRTPSPVHPTGTSQPQRPEDCRPRGSVKGTGLDFACDIYIWAPLAGICVALLLSLIITLICYHRQL
  CDS 1180..1593: note = murine CD3zeta ICD; protein_id = 64; translation = RRPGLTRKPYQPYAPARDFAAYRPRAKFSRSAETAANLQDPNQLYNELNLGRREEYDVLEKKRARDPEMGGKQQRRRNPQEGVYNALQKDKMAEAYSEIGTKGERRRGKGHDGLYQGLSTATKDTYDALHMQTLAPRS
  CDS 1594..1602: note = linker; translation = SRG
  CDS 1603..1659: note = P2A site; protein_id = 65; translation = ATNFSLLKQAGDVEENPGP
  misc_feature 554: note = DNA linker
  CDS 1663..2952: note = murine FOXP3; protein_id = 66; translation = MPNPRPAKPMAPSLALGPSPGVLPSWKTAPKGSELLGTRGSGGPFQGRDLRSGAHTSSSLNPLPPSQLQLPTVPLVMVAPSGARLGPSPHLQALLQDRPHFMHQLSTVDAHAQTPVLQVRPLDNPAMISLPPPSAATGVFSLKARPGLPPGINVASLEWVSREPALLCTFPRSGTPRKDSNLLAAPQGSYPLLANGVCKWPGCEKVFEEPEEFLKHCQADHLLDEKGKAQCLLQREVVQSLEQQLELEKEKLGAMQAHLAGKMALAKAPSVASMDKSSCCIVATSTQGSVLPAWSAPREAPDGGLFAVRRHLWGSHGNSSFPEFFHNMDYFKYHNMRPPFTYATLIRWAILEAPERQRTLNEIYHWFTRMFAYFRNHPATWKNAIRHNLSLHKCFVRVESEKGAVWTVDEFEFRKKRSQRPNKCSNPCP
  misc_feature 2953..2961: note = DNA linker
  primer_bind 2962..3533: note = IRES
  misc_feature 3534..3540: note = DNA linker
  CDS 3541..4032: note = Thy1.1; protein_id = 67; translation = MGNPAISVALLLSVLQVSRGQKVTSLTACLVNQNLRLDCRHENNTKDNSIQHEFSLTREKRKHVLSGTLGIPEHTYRSRVTLSNQPYIKVLTLANFTTKDEGDYFCELQVSGANPMSSNKSISVYRDKLVKCGGISLLVQNTSWMLLLLLSLSLLQALDFISL
  CDS 1660..1662: note = linker; translation = S
atgaaatacctattgcctacggcagccgctggcttgctgctgctggcagctcagccggccatggcccaggtgcagctgcaggagtcggggggaggcctggtcaagcctggggggtccctgagactctcctgtgcagcctctggattcaccttcagtagctatagcatgaactgggtccgccaggctccagggaaggggctggagtgggtctcatccattagtagtagtagttacatatactacgcagactcagtgaagggccgattcaccatctccagagacaacgccaagaactcgctgtatctgcaaatgaacagcctgagagccgaggacacggctgtgtattactgtgcgagacgggagggtggtaaatactactacggtatggacgtctggggccaagggaccacggtcaccgtctcctcagggagtgcatccgccccaaagcttgaagaaggtgaattttcagaagcacgcgtacagtctgccctgactcagcctccctccgcgtccgggtctcctggacagtcagtcaccatctcctgcactggaaccagcagtgacgtcggtgcctataactatgtctcctggtaccaacaacacccaggcaaagcccccaaactcatgatttatgaggtcactgagcggccctcaggggtccctgatcgcttctctggctccaagtctggcaacacggcctccctgaccatctctgggctccaggctgaggacgaggctgattattactgcagctcatatacaaccagtagcactgtgcttttcggcggagggaccaagctgaccgtcctaggtcagcccaaggctgccccctcggtcactctgttcccaccctcctctgcggccgcattcagctctgtggtgcccgtgctgcagaaagtgaacagcaccaccacaaagcctgtgctgagaaccccttctcctgtgcaccctaccggcacaagccagcctcaaagacctgaggactgcagacctagaggctccgtgaaaggcacaggcctggacttcgcctgcgacatctatatctgggctcctctggccggcatctgtgtggctctgctgctgagcctgatcatcaccctgatctgctaccacagacaattgtggaccaacagcagacggaacagactgctgcagagcgactacatgaacatgacccctagaaggcctggcctgaccagaaagccctaccagccttacgctcccgccagagatttcgccgcctacagaccaagagccaagttcagcagatccgccgagacagccgctaacctgcaggaccctaaccagctgtacaacgagctgaacctggggagaagagaagagtacgacgtgctggaaaagaagagagccagagatcccgagatgggaggcaagcagcagcggagaagaaaccctcaagagggcgtgtacaatgccctgcaaaaggacaagatggccgaggcctacagcgagatcggaactaagggcgagcgcagaagaggcaagggacacgatggactgtaccagggcctgagcacagccacaaaggacacatacgacgccctgcacatgcagacactggccccaagatcttctagaggagccaccaacttctccctgctgaagcaggccggcgacgtggaggagaaccccggcccctctatgcctaatcctagacctgccaagcctatggctcccagccttgctcttggaccttctccaggcgttctgcccagctggaaaacagcccctaagggctctgagctgctgggcacaagaggaagcggaggcccatttcagggacgcgatcttagatctggcgcccacacctcctccagcctgaatccacttcctccaagccagctccagctgcctacagtgccactggttatggtggcacctagcggagctagactgggaccctctccacatctgcaggctctgctccaggacagaccccactttatgcaccagctgagcaccgtggatgcccacgctcagacacctgttcttcaagtgcggcccctggacaaccccgctatgatttcactgcctcctccatctgccgccaccggcgttttcagtctgaaggctagacctggcctgcctcctggaatcaacgtggcctctctggaatgggtgtccagagaacccgctctgctgtgtacattccccagaagcggcacccctaggaaggactctaatctgctggctgctccccagggctcttaccctcttcttgctaacggcgtgtgcaagtggcctggctgcgaaaaggtgttcgaggaacccgaagagttcctgaagcactgccaggcagaccatctgctggacgagaagggcaaagctcagtgtctcctgcagcgcgaggtggtgcagtctctggaacagcagctggaactcgagaaagaaaagctgggcgccatgcaggctcacctggctggaaagatggctctggccaaggctccttctgtggccagcatggacaagagcagctgttgcatcgtggccacctctacacagggaagcgtgttgcctgcttggagcgcccctagagaagctcctgatggtggcctgtttgccgtgcggagacatctgtggggaagccacggcaactctagcttccccgagttcttccacaacatggactacttcaagtaccacaatatgcggcctccattcacctacgccacactgatcagatgggccatcctggaagcccctgagagacagagaacactgaacgagatctaccactggttcaccaggatgttcgcctacttcagaaatcaccccgccacctggaagaacgccatcagacacaacctgtctctgcacaagtgcttcgtgcgcgtggaatctgagaagggcgctgtgtggacagtggacgagttcgagttccgcaagaaaagaagccagaggccaaacaagtgcagcaacccctgtccttaatctagatgacccctctccctcccccccccctaacgttactggccgaagccgcttggaataaggccggtgtgcgtttgtctatatgttattttccaccatattgccgtcttttggcaatgtgagggcccggaaacctggccctgtcttcttgacgagcattcctaggggtctttcccctctcgccaaaggaatgcaaggtctgttgaatgtcgtgaaggaagcagttcctctggaagcttcttgaagacaaacaacgtctgtagcgaccctttgcaggcagcggaaccccccacctggcgacaggtgcctctgcggccaaaagccacgtgtataagatacacctgcaaaggcggcacaaccccagtgccacgttgtgagttggatagttgtggaaagagtcaaatggctctcctcaagcgtattcaacaaggggctgaaggatgcccagaaggtaccccattgtatgggatctgatctggggcctcggtgcacatgctttacatgtgtttagtcgaggttaaaaaacgtctaggccccccgaaccacggggacgtggtttccctttgaaaaacacgataatactccggaatgggaaacccagccatcagcgtcgctctcctgctctcagtcttgcaggtgtcccgagggcagaaggtgaccagcctgacagcctgcctggtgaaccaaaaccttcgcctggactgccgccatgagaataacaccaaggataactccatccagcatgagttcagcctgacccgagagaagaggaagcacgtgctctcaggcacccttgggatacccgagcacacgtaccgctcccgcgtcaccctctccaaccagccctatatcaaggtccttaccctagccaacttcaccaccaaggatgagggcgactacttttgtgagcttcaagtctcgggcgcgaatcccatgagctccaataaaagtatcagtgtgtatagagacaagctggtcaagtgtggcggcataagcctgctggttcagaacacatcctggatgctgctgctgctgctttccctctccctcctccaagccctggacttcatttctctgtga

SEQ ID NO: 42 - DNA, 4539 bp, synthetic construct
  source 1..4539: mol_type = other DNA
  CDS 1..864: note = secretory signal - scFv UK017-F8; protein_id = 68; translation = MKYLLPTAAAGLLLLAAQPAMAQVQLQESGGGLVKPGGSLRLSCAASGFTFSSYSMNWVRQAPGKGLEWVSSISSSSYIYYADSVKGRFTISRDNAKNSLYLQMNSLRAEDTAVYYCARREGGKYYYGMDVWGQGTTVTVSSGSASAPKLEEGEFSEARVQSALTQPPSASGSPGQSVTISCTGTSSDVGAYNYVSWYQQHPGKAPKLMIYEVTERPSGVPDRFSGSKSGNTASLTISGLQAEDEADYYCSSYTTSSTVLFGGGTKLTVLGQPKAAPSVTLFPPSSAA
  CDS 865..1551: note = murine IgG hinge; protein_id = 69; translation = ADPVPRDGGCKPCICTVPEVSSVFIFPPKPKDVLTITLTPKVTCVVVDISKDDPEVQFSWFVDDVEVHTAQTQPREEQFNSTFRSVSELPIMHQDWLNGKEFKCRVNSAAFPAPIEKTISKTKGRPKAPQVCTIPPPKEQMAKDKVSLTCMITDFFPEDITVEWQWNGQPAENYKNTQPIMDTDGSYFVYSKLNVQKSNWEAGNTFTCSVLHEGLHNHHTEKSLSHSPG
  CDS 1552..1557: note = linker; translation = QL
  CDS 1558..1686: note = murine CD8 ICD; protein_id = 70; translation = IVFLACVLGGSFGFLGFLGLCILCCVNSRRNRLLQSDYMNMTP
  CDS 1687..2100: note = murine CD3zeta ICD; protein_id = 71; translation = RRPGLTRKPYQPYAPARDFAAYRPLRAKFSRSAETAANLQDPNQLYNELNLGRREEYDVLEKKRARDPEMGGKQQRRRNPQEGVYNALQKDKMAEAYSEIGTKGERRRGKGHDGLYQGLSTATKDTYDALHMQTLAPR
  CDS 2101..2109: note = linker; translation = SRG
  CDS 2110..2166: note = P2A site; protein_id = 72; translation = ATNFSLLKQAGDVEENPGP
  CDS 2167..2169: note = linker; translation = S
  CDS 2170..3459: note = murine FoxP3; protein_id = 73; translation = MPNPRPAKPMAPSLALGPSPGVLPSWKTAPKGSELLGTRGSGGPFQGRDLRSGAHTSSSLNPLPPSQLQLPTVPLVMVAPSGARLGPSPHLQALLQDRPHFMHQLSTVDAHAQTPVLQVRPLDNPAMISLPPPSAATGVFSLKARPGLPPGINVASLEWVSREPALLCTFPRSGTPRKDSNLLAAPQGSYPLLANGVCKWPGCEKVFEEPEEFLKHCQADHLLDEKGKAQCLLQREVVQSLEQQLELEKEKLGAMQAHLAGKMALAKAPSVASMDKSSCCIVATSTQGSVLPAWSAPREAPDGGLFAVRRHLWGSHGNSSFPEFFHNMDYFKYHNMRPPFTYATLIRWAILEAPERQRTLNEIYHWFTRMFAYFRNHPATWKNAIRHNLSLHKCFVRVESEKGAVWTVDEFEFRKKRSQRPNKCSNPCP
  misc_feature 3460..3468: note = DNA linker
  primer_bind 3469..4040: note = IRES
  misc_feature 4041..4047: note = DNA linker
  CDS 4048..4539: note = Thy1.1; protein_id = 74; translation = MGNPAISVALLLSVLQVSRGQKVTSLTACLVNQNLRLDCRHENNTKDNSIQHEFSLTREKRKHVLSGTLGIPEHTYRSRVTLSNQPYIKVLTLANFTTKDEGDYFCELQVSGANPMSSNKSISVYRDKLVKCGGISLLVQNTSWMLLLLLSLSLLQALDFISL
atgaaatacctattgcctacggcagccgctggcttgctgctgctggcagctcagccggccatggcccaggtgcagctgcaggagtcggggggaggcctggtcaagcctggggggtccctgagactctcctgtgcagcctctggattcaccttcagtagctatagcatgaactgggtccgccaggctccagggaaggggctggagtgggtctcatccattagtagtagtagttacatatactacgcagactcagtgaagggccgattcaccatctccagagacaacgccaagaactcgctgtatctgcaaatgaacagcctgagagccgaggacacggctgtgtattactgtgcgagacgggagggtggtaaatactactacggtatggacgtctggggccaagggaccacggtcaccgtctcctcagggagtgcatccgccccaaagcttgaagaaggtgaattttcagaagcacgcgtacagtctgccctgactcagcctccctccgcgtccgggtctcctggacagtcagtcaccatctcctgcactggaaccagcagtgacgtcggtgcctataactatgtctcctggtaccaacaacacccaggcaaagcccccaaactcatgatttatgaggtcactgagcggccctcaggggtccctgatcgcttctctggctccaagtctggcaacacggcctccctgaccatctctgggctccaggctgaggacgaggctgattattactgcagctcatatacaaccagtagcactgtgcttttcggcggagggaccaagctgaccgtcctaggtcagcccaaggctgccccctcggtcactctgttcccaccctcctctgcggccgcagatcccgttcctcgagatggcggatgcaagccctgcatctgtaccgtgcctgaggtgtccagcgtgttcatcttcccacctaagcctaaggacgtgctgacaatcaccctgacacctaaagtgacctgcgtggtggtggacatcagcaaggacgatcccgaggtgcagttcagttggttcgtggacgacgtggaagtgcacaccgctcagacacagcccagagaggaacagttcaactccaccttcagatctgtgtccgagctgcccatcatgcaccaggattggctgaacggcaaagaattcaagtgccgcgtgaactccgccgcctttcctgctcctatcgaaaagaccatctccaagaccaagggcagacccaaggctccccaagtgtgcacaatccctccacctaaagaacagatggccaaggacaaggtgtccctgacctgcatgatcaccgatttcttcccagaggacatcaccgtggaatggcagtggaacggacagcccgccgagaactacaagaacacccagcctatcatggacaccgacggcagctacttcgtgtacagcaagctgaacgtgcagaagtccaactgggaggccggcaacacctttacctgtagcgtgctgcacgagggcctgcacaaccaccacacagagaagtctctgagccactctcctggccaattgatcgtgttcctggcctgtgtgctcggcggctcttttggcttcctgggctttctgggcctgtgcatcctgtgctgcgtgaacagcagaagaaacagactgctgcagagcgactacatgaacatgacccctagaaggcctggcctgacaagaaagccctaccagccttacgctcccgccagagatttcgccgcttacagacctctgagagccaagttctccagaagcgccgagacagccgctaacctgcaggaccctaaccagctgtacaacgagctgaacctggggagaagagaagagtacgacgtgctggaaaagaagagagccagagatcccgagatgggaggcaagcagcagagaagaagaaaccctcaagagggcgtgtacaatgccctgcagaaagacaagatggccgaggcctacagcgagatcggaactaagggcgaacgcagaagaggcaagggccacgatggactgtaccagggactgagcacagccaccaaggacacatacgacgccctgcacatgcagacactggcccctaggtctagaggagccaccaacttctccctgctgaagcaggccggcgacgtggaggagaaccccggcccctctatgcctaatcctagacctgccaagcctatggctcccagccttgctcttggaccttctcctggcgttctgcccagctggaaaacagcccctaagggctctgagctgctgggcacaagaggaagcggaggcccatttcagggacgcgatcttagatctggcgcccacacctcctccagcctgaatccacttcctccaagccagctccagctgcctacagtgccactggttatggtggcacctagcggagctagactgggaccctctccacatctgcaggctctgctgcaggacagaccccactttatgcaccagctgagcaccgtggatgcccacgctcaaacaccagtgctgcaagtccggcctctggacaaccccgctatgatctcactgcctcctccatctgctgccaccggcgtgttcagcctgaaagctagacctggactgcctccaggcatcaacgtggcatctctggaatgggtgtcccgcgaacctgctctgctgtgcacatttcccagaagcggcacccctaggaaggacagcaatctgctggctgctccccagggctcttatcctctgcttgctaacggcgtgtgcaagtggcctggatgcgagaaggtgttcgaggaacccgaagagttcctgaagcactgccaggctgatcatctgctggacgagaagggcaaagcccagtgtctcctgcagagagaggtggtccagagcctggaacagcagctggaactcgagaaagaaaagctgggcgccatgcaggctcacctggctggaaaaatggccctggctaaggcccctagcgtggccagcatggacaagagcagctgttgtatcgtggccacctccacacagggatctgtgttgcctgcttggagcgcccctagagaagctcctgatggtggcctgtttgccgtgcggagacatctgtggggaagccacggcaactctagcttccccgagttcttccacaacatggactacttcaagtaccacaatatgcggcctccattcacctacgccacactgatcagatgggccatcctggaagcccctgagagacagagaaccctgaacgagatctaccactggttcaccagaatgttcgcctacttcagaaatcaccccgccacctggaagaacgccatcagacacaacctgtctctgcacaagtgcttcgtgcgcgtggaatctgagaagggcgctgtgtggacagtggacgagttcgagttccgcaagaagagatcccagaggccaaacaagtgcagcaacccctgtccttaatctagatgacccctctccctcccccccccctaacgttactggccgaagccgcttggaataaggccggtgtgcgtttgtctatatgttattttccaccatattgccgtcttttggcaatgtgagggcccggaaacctggccctgtcttcttgacgagcattcctaggggtctttcccctctcgccaaaggaatgcaaggtctgttgaatgtcgtgaaggaagcagttcctctggaagcttcttgaagacaaacaacgtctgtagcgaccctttgcaggcagcggaaccccccacctggcgacaggtgcctctgcggccaaaagccacgtgtataagatacacctgcaaaggcggcacaaccccagtgccacgttgtgagttggatagttgtggaaagagtcaaatggctctcctcaagcgtattcaacaaggggctgaaggatgcccagaaggtaccccattgtatgggatctgatctggggcctcggtgcacatgctttacatgtgtttagtcgaggttaaaaaacgtctaggccccccgaaccacggggacgtggtttccctttgaaaaacacgataatactccggaatgggaaacccagccatcagcgtcgctctcctgctctcagtcttgcaggtgtcccgagggcagaaggtgaccagcctgacagcctgcctggtgaaccaaaaccttcgcctggactgccgccatgagaataacaccaaggataactccatccagcatgagttcagcctgacccgagagaagaggaagcacgtgctctcaggcacccttgggatacccgagcacacgtaccgctcccgcgtcaccctctccaaccagccctatatcaaggtccttaccctagccaacttcaccaccaaggatgagggcgactacttttgtgagcttcaagtctcgggcgcgaatcccatgagctccaataaaagtatcagtgtgtatagagacaagctggtcaagtgtggcggcataagcctgctggttcagaacacatcctggatgctgctgctgctgctttccctctccctcctccaagccctggacttcatttctctgtga

SEQ ID NO: 43 - protein, 280 aa, synthetic construct; identical to SEQ ID NO: 2

SEQ ID NO: 44 - protein, 231 aa, synthetic construct
EPKSPDKTHTCPPCPAPPVAGPSVFLFPPKPKDTLMIARTPEVTCVVVDVSHEDPEVKFNWYVDGVEVHNAKTKPREEQYNSTYRVVSVLTVLHQDWLNGKEYKCKVSNKALPAPIEKTISKAKGQPREPQVYTLPPSRDELTKNQVSLTCLVKGFYPSDIAVEWESNGQPENNYKTTPPVLDSDGSFFLYSKLTVDKSRWQQGNVFSCSVMHEALHNHYTQKSLSLSPGK

SEQ ID NO: 45 - protein, 33 aa, synthetic construct
KQLDPKFWVLVVVGGVLACYSLLVTVAFIIFWV

SEQ ID NO: 46 - protein, 41 aa, synthetic construct
RSKRSRLLHSDYMNMTPRRPGPTRKHYQAYAAARDFAAYRS

SEQ ID NO: 47 - protein, 112 aa, synthetic construct; identical to SEQ ID NO: 34

SEQ ID NO: 48 - protein, 19 aa, synthetic construct
ATNFSLLKQAGDVEENPGP

SEQ ID NO: 49 - protein, 431 aa, synthetic construct; identical to SEQ ID NO: 38

SEQ ID NO: 50 - protein, 280 aa, synthetic construct
MGAGATGRAMDGPRLLLLLLLGVSLGGAKEACPTGLYTHSGECCKACNLGEGVAQPCGANQTVCEPCLDSVTFSDVVSATEPCKPCTECVGLQSMSAPCVEADDAVCRCAYGYYQDETTGRCEACRVCEAGSGLVFSCQDKQNTVCEECPDGTYSDEANHVDPCLPCTVCEDTERQLRECTRWADAECEEIPGRWITRSTPPEGSDSTAPSTQEPEAPPEQDLIASTVAGVVTTVMGSSQPVVTRGTTDNLIPVYCSILAAVVVGLVAYIAFKRWNRGIL

SEQ ID NO: 51 - protein, 280 aa, synthetic construct; identical to SEQ ID NO: 2

SEQ ID NO: 52 - protein, 53 aa, synthetic construct
FVPVFLPAKPTTTPAPRPPTPAPTIASQPLSLRPEASRPAAGGAVHTRGLDFA

SEQ ID NO: 53 - protein, 28 aa, synthetic construct
DIYIWAPLAGTCGVLLLSLVITLYCNHR

SEQ ID NO: 54 - protein, 4 aa, synthetic construct
QLWV

SEQ ID NO: 55 - protein, 41 aa, synthetic construct
RSKRSRLLHSDYMNMTPRRPGPTRKHYQPYAPPRDFAAYRS

SEQ ID NO: 56 - protein, 112 aa, synthetic construct; identical to SEQ ID NO: 34

SEQ ID NO: 57 - protein, 4 aa, synthetic construct
SSRG

SEQ ID NO: 58 - protein, 19 aa, synthetic construct
ATNFSLLKQAGDVEENPGP

SEQ ID NO: 59 - protein, 431 aa, synthetic construct; identical to SEQ ID NO: 38

SEQ ID NO: 60 - protein, 281 aa, synthetic construct
GMGAGATGRAMDGPRLLLLLLLGVSLGGAKEACPTGLYTHSGECCKACNLGEGVAQPCGANQTVCEPCLDSVTFSDVVSATEPCKPCTECVGLQSMSAPCVEADDAVCRCAYGYYQDETTGRCEACRVCEAGSGLVFSCQDKQNTVCEECPDGTYSDEANHVDPCLPCTVCEDTERQLRECTRWADAECEEIPGRWITRSTPPEGSDSTAPSTQEPEAPPEQDLIASTVAGVVTTVMGSSQPVVTRGTTDNLIPVYCSILAAVVVGLVAYIAFKRWNRGIL

SEQ ID NO: 61 - protein, 288 aa, synthetic construct; identical to SEQ ID NO: 12

SEQ ID NO: 62 - protein, 19 aa, synthetic construct
WTNSRRNRLLQSDYMNMTP

SEQ ID NO: 63 - protein, 86 aa, synthetic construct
AFSSVVPVLQKVNSTTTKPVLRTPSPVHPTGTSQPQRPEDCRPRGSVKGTGLDFACDIYIWAPLAGICVALLLSLIITLICYHRQL

SEQ ID NO: 64 - protein, 138 aa, synthetic construct
RRPGLTRKPYQPYAPARDFAAYRPRAKFSRSAETAANLQDPNQLYNELNLGRREEYDVLEKKRARDPEMGGKQQRRRNPQEGVYNALQKDKMAEAYSEIGTKGERRRGKGHDGLYQGLSTATKDTYDALHMQTLAPRS

SEQ ID NO: 65 - protein, 19 aa, synthetic construct
ATNFSLLKQAGDVEENPGP

SEQ ID NO: 66 - protein, 429 aa, synthetic construct; identical to SEQ ID NO: 36

SEQ ID NO: 67 - protein, 163 aa, synthetic construct
MGNPAISVALLLSVLQVSRGQKVTSLTACLVNQNLRLDCRHENNTKDNSIQHEFSLTREKRKHVLSGTLGIPEHTYRSRVTLSNQPYIKVLTLANFTTKDEGDYFCELQVSGANPMSSNKSISVYRDKLVKCGGISLLVQNTSWMLLLLLSLSLLQALDFISL

SEQ ID NO: 68 - protein, 288 aa, synthetic construct; identical to SEQ ID NO: 12

SEQ ID NO: 69 - protein, 229 aa, synthetic construct
ADPVPRDGGCKPCICTVPEVSSVFIFPPKPKDVLTITLTPKVTCVVVDISKDDPEVQFSWFVDDVEVHTAQTQPREEQFNSTFRSVSELPIMHQDWLNGKEFKCRVNSAAFPAPIEKTISKTKGRPKAPQVCTIPPPKEQMAKDKVSLTCMITDFFPEDITVEWQWNGQPAENYKNTQPIMDTDGSYFVYSKLNVQKSNWEAGNTFTCSVLHEGLHNHHTEKSLSHSPG

SEQ ID NO: 70 - protein, 43 aa, synthetic construct
IVFLACVLGGSFGFLGFLGLCILCCVNSRRNRLLQSDYMNMTP

SEQ ID NO: 71 - protein, 138 aa, synthetic construct
RRPGLTRKPYQPYAPARDFAAYRPLRAKFSRSAETAANLQDPNQLYNELNLGRREEYDVLEKKRARDPEMGGKQQRRRNPQEGVYNALQKDKMAEAYSEIGTKGERRRGKGHDGLYQGLSTATKDTYDALHMQTLAPR

SEQ ID NO: 72 - protein, 19 aa, synthetic construct
ATNFSLLKQAGDVEENPGP

SEQ ID NO: 73 - protein, 429 aa, synthetic construct; identical to SEQ ID NO: 36

SEQ ID NO: 74 - protein, 163 aa, synthetic construct; identical to SEQ ID NO: 67